European Patent Specification EP 3 062 802 B1, published November 15, 2023. Title: EXTRACTS FROM PLANTS OF THE MORINGACEAE FAMILY AND METHODS OF MAKING. Applicant: Raskin, et al. The sequence listing filed with the application follows.

SEQUENCE LISTING (12 sequences)

SEQ ID NO: 1 - DNA, 23 bp, Artificial Sequence
  Synthetic primer
aaccgtgaaaagatgacccagat

SEQ ID NO: 2 - DNA, 20 bp, Artificial Sequence
  Synthetic primer
cacagcctggatggctacgt

SEQ ID NO: 3 - DNA, 24 bp, Artificial Sequence
  Synthetic primer
caaccaacaagtgatattctccat

SEQ ID NO: 4 - DNA, 21 bp, Artificial Sequence
  Synthetic primer
gatccacactctccagctgca

SEQ ID NO: 5 - DNA, 21 bp, Artificial Sequence
  Synthetic primer
ccctcctgatcttgtgttgga

SEQ ID NO: 6 - DNA, 19 bp, Artificial Sequence
  Synthetic primer
tcaacccgagctcctggaa

SEQ ID NO: 7 - DNA, 20 bp, Artificial Sequence
  Synthetic primer
tggtgcctggtctgatgatg

SEQ ID NO: 8 - DNA, 21 bp, Artificial Sequence
  Synthetic primer
gtggtaaccgctcaggtgttg

SEQ ID NO: 9 - DNA, 23 bp, Artificial Sequence
  Synthetic primer
tgggagtagacaaggtacaaccc

SEQ ID NO: 10 - DNA, 25 bp, Artificial Sequence
  Synthetic primer
catcttctcaaaattcgagtgagaa

SEQ ID NO: 11 - DNA, 24 bp, Artificial Sequence
  Synthetic primer
tcggaggcttaattacacatgttc

SEQ ID NO: 12 - DNA, 22 bp, Artificial Sequence
  Synthetic primer
tgccattgcacaactcttttct